European Patent Specification EP 4 036 104 B1, published February 21, 2024. Title: Factor H Binding Proteins (FHBP) with Altered Properties and Methods of Use Thereof. Applicant: Childrens Hospital and Research Center Oakland. Application EP. The sequence listing filed with the application follows.

SEQUENCE LISTING (31 sequences)

SEQ ID NO: 1 - protein, 255 aa, Neisseria meningitidis
CSSGGGGVAADIGAGLADALTAPLDHKDKGLQSLTLDQSVRKNEKLKLAAQGAEKTYGNGDSLNTGKLKNDKVSRFDFIRQIEVDGQLITLESGEFQVYKQSHSALTAFQTEQIQDSEHSGKMVAKRQFRIGDIAGEHTSFDKLPEGGRATYRGTAFGSDDAGGKLTYTIDFAAKQGNGKIEHLKSPELNVDLAAADIKPDGKRHAVISGSVLYNQAEKGSYSLGIFGGKAQEVAGSAEVKTVNGIRHIGLAAKQ

SEQ ID NO: 2 - protein, 254 aa, Neisseria meningitidis
CSSGGGGVAADIGAGLADALTAPLDHKDKSLQSLTLDQSVRKNEKLKLAAQGAEKTYGNGDSLNTGKLKNDKVSRFDFIRQIEVDGQLITLESGEFQIYKQDHSAVVALQIEKINNPDKIDSLINQRSFLVSGLGGEHTAFNQLPSGKAEYHGKAFSSDDPNGRLHYSIDFTKKQGYGRIEHLKTPEQNVELASAELKADEKSHAVILGDTRYGGEEKGTYHLALFGDRAQEIAGSATVKIREKVHEIGIAGKQ

SEQ ID NO: 3 - protein, 262 aa, Neisseria meningitidis
CSSGGGGSGGGGVAADIGTGLADALTAPLDHKDKGLKSLTLEDSIPQNGTLTLSAQGAEKTFKAGDKDNSLNTGKLKNDKISRFDFVQKIEVDGQTITLASGEFQIYKQNHSAVVALQIEKINNPDKTDSLINQRSFLVSGLGGEHTAFNQLPGGKAEYHGKAFSSDDPNGRLHYSIDFTKKQGYGRIEHLKTLEQNVELAAAELKADEKSHAVILGDTRYGSEEKGTYHLALFGDRAQEIAGSATVKIGEKVHEIGIAGKQ

SEQ ID NO: 4 - protein, 254 aa, Neisseria meningitidis
CSSGGGGVAADIGARLADALTAPLDHKDKSLQSLTLDQSVRKNEKLKLAAQGAEKTYGNGDSLNTGKLKNDKVSRFDFIRQIEVDGQLITLESGEFQIYKQDHSAVVALQIEKINNPDKIDSLINQRSFLVSGLGGEHTAFNQLPDGKAEYHGKAFSSDDAGGKLTYTIDFAAKQGHGKIEHLKTPEQNVELAAAELKADEKSHAVILGDTRYGSEEKGTYHLALFGDRAQEIAGSATVKIGEKVHEIGIAGKQ

SEQ ID NO: 5 - protein, 263 aa, Neisseria meningitidis
CSSGGGGSGGGGVAADIGAGLADALTAPLDHKDKGLKSLTLEDSISQNGTLTLSAQGAERTFKAGDKDNSLNTGKLKNDKISRFDFIRQIEVDGQLITLESGEFQVYKQSHSALTALQTEQVQDSEHSGKMVAKRQFRIGDIVGEHTSFGKLPKDVMATYRGTAFGSDDAGGKLTYTIDFAAKQGHGKIEHLKSPELNVDLAAADIKPDEKHHAVISGSVLYNQAEKGSYSLGIFGGQAQEVAGSAEVETANGIRHIGLAAKQ

SEQ ID NO: 6 - protein, 255 aa, Neisseria meningitidis
CSSGGGGVAADIGAGLADALTAPLDHKDKGLQSLTLDQSVRKNEKLKLAAQGAEKTYGNGDSLNTGKLKNDKVSRFDFIRQIEVNGQLITLESGEFQVYKQSHSALTALQTEQVQDSEHSRKMVAKRQFRIGDIAGEHTSFDKLPKGDSATYRGTAFGSDDAGGKLTYTIDFAAKQGYGKIEHLKSPELNVDLAAAYIKPDEKHHAVISGSVLYNQDEKGSYSLGIFGGQAQEVAGSAEVKTANGIRHIGLAAKQ

SEQ ID NO: 7 - protein, 255 aa, Neisseria meningitidis
CSSGGGGVAADIGAGLADALTAPLDHKDKSLQSLTLDQSVRKNEKLKLAAQGAEKTYGNGDSLNTGKLKNDKVSRFDFIRQIEVDGQLITLESGEFQVYKQSHSALTALQTEQEQDPEHSGKMVAKRRFKIGDIAGEHTSFDKLPKDVMATYRGTAFGSDDAGGKLTYTIDFAAKQGHGKIEHLKSPELNVELATAYIKPDEKHHAVISGSVLYNQDEKGSYSLGIFGGQAQEVAGSAEVETANGIHHIGLAAKQ

SEQ ID NO: 8 - protein, 254 aa, Artificial Sequence
  Chimera fHbp ID 1 and ID 77
CSSGGGGVAADIGAGLADALTAPLDHKDKGLQSLTLDQSVRKNEKLKLAAQGAEKTYGNGDSLNTGKLKNDKVSRFDFIRQIEVDGQLITLESGEFQVYKQSHSALTAFQTEQIQDSEHSGKMVAKRQFRIGDIAGEHTAFNQLPDGKAEYHGKAFSSDDAGGKLTYTIDFAAKQGHGKIEHLKTPEQNVELAAAELKADEKSHAVILGDTRYGSEEKGTYHLALFGDRAQEIAGSATVKIGEKVHEIGIAGKQ

SEQ ID NO: 9 - protein, 1231 aa, Homo sapiens
MRLLAKIICLMLWAICVAEDCNELPPRRNTEILTGSWSDQTYPEGTQAIYKCRPGYRSLGNVIMVCRKGEWVALNPLRKCQKRPCGHPGDTPFGTFTLTGGNVFEYGVKAVYTCNEGYQLLGEINYRECDTDGWTNDIPICEVVKCLPVTAPENGKIVSSAMEPDREYHFGQAVRFVCNSGYKIEGDEEMHCSDDGFWSKEKPKCVEISCKSPDVINGSPISQKIIYKENERFQYKCNMGYEYSERGDAVCTESGWRPLPSCEEKSCDNPYIPNGDYSPLRIKHRTGDEITYQCRNGFYPATRGNTAKCTSTGWIPAPRCTLKPCDYPDIKHGGLYHENMRRPYFPVAVGKYYSYYCDEHFETPSGSYWDHIHCTQDGWSPAVPCLRKCYFPYLENGYNQNYGRKFVQGKSIDVACHPGYALPKAQTTVTCMENGWSPTPRCIRVKTCSKSSIDIENGFISESQYTYALKEKAKYQCKLGYVTADGETSGSITCGKDGWSAQPTCIKSCDIPVFMNARTKNDFTWFKLNDTLDYECHDGYESNTGSTTGSIVCGYNGWSDLPICYERECELPKIDVHLVPDRKKDQYKVGEVLKFSCKPGFTIVGPNSVQCYHFGLSPDLPICKEQVQSCGPPPELLNGNVKEKTKEEYGHSEVVEYYCNPRFLMKGPNKIQCVDGEWTTLPVCIVEESTCGDIPELEHGWAQLSSPPYYYGDSVEFNCSESFTMIGHRSITCIHGVWTQLPQCVAIDKLKKCKSSNLIILEEHLKNKKEFDHNSNIRYRCRGKEGWIHTVCINGRWDPEVNCSMAQIQLCPPPPQIPNSHNMTTTLNYRDGEKVSVLCQENYLIQEGEEITCKDGRWQSIPLCVEKIPCSQPPQIEHGTINSSRSSQESYAHGTKLSYTCEGGFRISEENETTCYMGKWSSPPQCEGLPCKSPPEISHGVVAHMSDSYQYGEEVTYKCFEGFGIDGPAIAKCLGEKWSHPPSCIKTDCLSLPSFENAIPMGEKKDVYKAGEQVTYTCATYYKMDGASNVTCINSRWTGRPTCRDTSCVNPPTVQNAYIVSRQMSKYPSGERVRYQCRSPYEMFGDEEVMCLNGNWTEPPQCKDSTGKCGPPPPIDNGDITSFPLSVYAPASSVEYQCQNLYQLEGNKRITCRNGQWSEPPKCLHPCVISREIMENYNIALRWTAKQKLYSRTGESVEFVCKRGYRLSSRSHTLRTTCWDGKLEYPTCAKR

SEQ ID NO: 10 - protein, 50 aa, Artificial Sequence
  Synthetic polypeptide
TAPLDHKDKGLQSLTLDQSVRKNEKLKLAAQGAEKTYGNGDSLNTGKLKN

SEQ ID NO: 11 - protein, 50 aa, Artificial Sequence
  Synthetic polypeptide
TAPLDHKDKSLQSLTLDQSVRKNEKLKLAAQGAEKTYGNGDSLNTGKLKN

SEQ ID NO: 12 - protein, 53 aa, Artificial Sequence
  Synthetic polypeptide
TAPLDHKDKGLKSLTLEDSISQNGTLTLSAQGAERTFKAGDKDNSLNTGKLKN

SEQ ID NO: 13 - protein, 50 aa, Artificial Sequence
  Synthetic polypeptide
TAPLDHKDKGLKSLTLEDSISQNGTLTLSAQGAEKTYGNGDSLNTGKLKN

SEQ ID NO: 14 - protein, 53 aa, Artificial Sequence
  Synthetic polypeptide
TAPLDHKDKGLKSLTLEDSIPQNGTLTLSAQGAEKTFKAGDKDNSLNTGKLKN

SEQ ID NO: 15 - protein, 174 aa, Neisseria meningitidis
MKKALATLIALALPAAALAEGASGFYVQADAAHAKASSSLGSAKGFSPRISAGYRINDLRFAVDYTRYKNYKAPSTDFKLYSIGASAIYDFDTQSPVKPYLGARLSLNRASVDLGGSDSFSQTSIGLGVLTGVSYAVTPNVDLDAGYRYNYIGKVNTVKNVRSGELSVGVRVKF

SEQ ID NO: 16 - protein, 19 aa, Artificial Sequence
  Synthetic polypeptide
MNRTAFCCLSLTTALILTA

SEQ ID NO: 17 - protein, 66 aa, Artificial Sequence
  Synthetic polypeptide
VAADIGAGLADALTAPLDHKDKSLQSLTLDQSVRKNEKLKLAAQGAEKTYGNGDSLNTGKLKNDKV

SEQ ID NO: 18 - protein, 5 aa, Artificial Sequence
  Synthetic polypeptide
FLLAV

SEQ ID NO: 19 - protein, 5 aa, Artificial Sequence
  Synthetic polypeptide
GSGGS

SEQ ID NO: 20 - protein, 4 aa, Artificial Sequence
  Synthetic polypeptide
GGGS

SEQ ID NO: 21 - protein, 4 aa, Artificial Sequence
  Synthetic polypeptide
GGSG

SEQ ID NO: 22 - protein, 5 aa, Artificial Sequence
  Synthetic polypeptide
GGSGG

SEQ ID NO: 23 - protein, 5 aa, Artificial Sequence
  Synthetic polypeptide
GSGSG

SEQ ID NO: 24 - protein, 5 aa, Artificial Sequence
  Synthetic polypeptide
GSGGG

SEQ ID NO: 25 - protein, 5 aa, Artificial Sequence
  Synthetic polypeptide
GGGSG

SEQ ID NO: 26 - protein, 5 aa, Artificial Sequence
  Synthetic polypeptide
GSSSG

SEQ ID NO: 27 - protein, 4 aa, Artificial Sequence
  Synthetic polypeptide
GEHT

SEQ ID NO: 28 - protein, 66 aa, Artificial Sequence
  Synthetic polypeptide
VAADIGAGLADALTAPLDHKDKGLQSLTLDQSVRKNEKLKLAAQGAEKTYGNGDSLNTGKLKNDKV

SEQ ID NO: 29 - protein, 66 aa, Artificial Sequence
  Synthetic polypeptide
VAADIGARLADALTAPLDHKDKSLQSLTLDQSVRKNEKLKLAAQGAEKTYGNGDSLNTGKLKNDKV

SEQ ID NO: 30 - protein, 60 aa, Artificial Sequence
  Synthetic polypeptide
VYKQSHSALTAFQTEQIQDSEHSGKMVAKRQFRIGDIAGEHTSFDKLPEGGRATYRGTAF

SEQ ID NO: 31 - protein, 60 aa, Artificial Sequence
  Synthetic polypeptide
VYKQSHSALTALQTEQVQDSEHSGKMVAKRQFRIGDIVGEHTSFGKLPKDVMATYRGTAF